European Patent Application EP 4 644 542 A1, published November 5, 2025. Title: Mutant allulose-3-epimerase and use thereof. Applicant: SAMYANG CORPORATION. The sequence listing filed with the application follows.

SEQUENCE LISTING (14 sequences)

SEQ ID NO: 1 - protein, 289 aa, synthetic construct
  REGION 1..289: note = MDPE_Wild_AA
MNIGCHGLVWTGHFDADGIRLSAEQTKAAGFDLIEFPLMDPFTFDVAAAKEALEEHDLAVSASLGLSGATDVTSSDPAVVAAGEALLMKAVDVLAELGGRHFCGVIYSAMQKYMDPVTTEGLESSRRTIARVADHAAERGISVSLEVVNRYETNVLNTARQALAYLAEVDRPNLGIHLDTYHMNIEESDMFAPVLDAAPALRYVHIGESHRGYLGTGTVDFDNFFKALGRIGYDGPIVFESFSSAVVAPDLSRMLGIWRNLWTDNVELGAHANAYIRDKLVAVDSIRLH

SEQ ID NO: 2 - DNA, 867 bp, synthetic construct
  misc_feature 1..867: note = MDPE_Wild_DNA
  source 1..867: mol_type = other DNA
atgaacatcggttgccacggtctggtttggaccggtcacttcgacgcggacggtatccgtctgtctgcggaacagaccaaagcggcgggtttcgacctgatcgaattcccgctgatggacccgttcaccttcgacgttgcggcggcgaaagaagcgctggaagaacacgacctggcggtttctgcgtctctgggtctgtctggtgcgaccgacgttacctcttctgacccggcggttgttgcggcgggtgaagcgctgctgatgaaagcggttgacgttctggcggaactgggtggtcgtcacttctgcggtgttatctactctgcgatgcagaaatacatggacccggttaccaccgaaggtctggaatcttctcgtcgtaccatcgcgcgtgttgcggaccacgcggcggaacgtggtatctctgtttctctggaagttgttaaccgttacgaaaccaacgttctgaacaccgcgcgtcaggcgctggcgtacctggcggaagttgaccgtccgaacctgggtatccacctggacacctaccacatgaacatcgaagaatctgacatgttcgcgccggttctggacgcggcgccggcgctgcgttacgttcacatcggtgaatctcaccgtggttacctgggtaccggtaccgttgacttcgacaacttcttcaaagcgctgggtcgtatcggttacgacggtccgatcgttttcgaatctttctcttctgcggttgttgcgccggacctgtctcgtatgctgggtatctggcgtaacctgtggaccgacaacgttgaactgggtgcgcacgcgaacgcgtacatccgtgacaaactggttgcggttgactctatccgtctgcac

SEQ ID NO: 3 - DNA, 38 bp, synthetic construct
  misc_feature 1..38: note = MDPE_Cloning_For_Primer
  source 1..38: mol_type = other DNA
ccatgattacgccaagcttatgaacatcggttgccacg

SEQ ID NO: 4 - DNA, 50 bp, synthetic construct
  misc_feature 1..50: note = MDPE_Cloning_Rev_Primer
  source 1..50: mol_type = other DNA
cggtacccggggatcctagcagccggatctcagtgcagacggatagagtc

SEQ ID NO: 5 - DNA, 38 bp, synthetic construct
  misc_feature 1..38: note = MDPE_A23I_Cloning_For_Primer
  source 1..38: mol_type = other DNA
gacggtatccgtctgtctattgaacagaccaaagcggc

SEQ ID NO: 6 - DNA, 38 bp, synthetic construct
  misc_feature 1..38: note = MDPE_A23I_Cloning_Rev_Primer
  source 1..38: mol_type = other DNA
gccgctttggtctgttcaatagacagacggataccgtc

SEQ ID NO: 7 - DNA, 33 bp, synthetic construct
  misc_feature 1..33: note = MDPE_S75E_Cloning_For_Primer
  source 1..33: mol_type = other DNA
cgaccgacgttacctctgaagacccggcggttg

SEQ ID NO: 8 - DNA, 33 bp, synthetic construct
  misc_feature 1..33: note = MDPE_S75E_Cloning_Rev_Primer
  source 1..33: mol_type = other DNA
caaccgccgggtcttcagaggtaacgtcggtcg

SEQ ID NO: 9 - DNA, 24 bp, synthetic construct
  misc_feature 1..24: note = MDPE_Mut_For_Primer
  source 1..24: mol_type = other DNA
gaccatgattacgccaagcttatg

SEQ ID NO: 10 - DNA, 35 bp, synthetic construct
  misc_feature 1..35: note = MDPE_Mut_Rev_Primer
  source 1..35: mol_type = other DNA
cggtacccggggatcctagcagccggatctcagtg

SEQ ID NO: 11 - DNA, 22 bp, synthetic construct
  misc_feature 1..22: note = M13F_Primer
  source 1..22: mol_type = other DNA
gcggataacaatttcacacagg

SEQ ID NO: 12 - DNA, 17 bp, synthetic construct
  misc_feature 1..17: note = M13R_Primer
  source 1..17: mol_type = other DNA
gtaaaacgacggccagt

SEQ ID NO: 13 - DNA, 40 bp, synthetic construct
  misc_feature 1..40: note = Enz_Cloning_For_Primer
  source 1..40: mol_type = other DNA
ctttaagaaggagatatacatatgaacatcggttgccacg

SEQ ID NO: 14 - DNA, 46 bp, synthetic construct
  misc_feature 1..46: note = Enz_Cloning_Rev_Primer
  source 1..46: mol_type = other DNA
ggtggtggtgctcgagtgcggccgcgtgcagacggatagagtcaac